European Patent Specification EP 3 462 904 B1, published December 18, 2024. Title: POLYPEPTIDES HAVING ALPHA-GALACTOSIDASE ACTIVITY AND POLYNUCLEOTIDES ENCODING SAME. Applicant: Novozymes A/S. The sequence listing filed with the application follows.

SEQUENCE LISTING (4 sequences)

SEQ ID NO: 1 - DNA, 2364 bp, Penicillium pseudopulvillorum
  CDS (1)..(82)
  sig_peptide (1)..(63)
  mat_peptide (64)..(2361)
  CDS (143)..(746)
  CDS (822)..(2361)
atgcagaaagcggttgcgagcgctagcttgctagccctgctcggctccacgtcggcagtggcagctcaaagcttttccaatggtcagttgcccttcttgagtactcttactgatccgcatactcatactcattcttcagcagtcgttgtggatggcaccaccttcgcactgaacggtgacaatttctcctaccgttttcatgtcgataacgagactggcgatctttggtcagaccacttcggtgcgagcgtgacaggcgatataccttttgagaatgttcctgccgtcaatggctgggtcggcatgccaggccgtgtccgtcgagaatttcctgaccagggccggggtgacttccgtattcctgccattcgtattcgacagtccgagggctatacagtctccgacttgcagtatcaatcgtacgatgtgatccaaggcaagcctgaactgccaggactgcccgctacttttggtaccgataaggatgtgacaaccttggtcgtccacctttatgataattatagtgccgtggcagcggatttgtcgtattccgtattccccaaatacgatgcgattgtccgcagtgtgaatgttaccaacaaaggccaggacaacattactattgaagcgctggctagtttgagtgtcgactttccctatcaagacttggacatgatcagcttgaggggtgattgggcccgggaagctcaccgcgagcgaagaaaagtcgagtacggaatacaagggtaagcctaacatacacccacagtgatctacagcgttgagggagaactgacatacgattgttgtcttgggattagatttggcagctctacgggatactcatcacacctccacaacccattccttgctcttgtcgatccaagtgccacagaatccagtggcgaagcgtggggcttctcgttagtgtataccggttcattttcggtggacgtcgagaaaggctctcagggcttcactcgtgctctacttggactcaatcccaaccagctctcttggaacctcggtaccggcgaaacgataaccacgcctgaatgcgtgtcggtctattcccagaatggagtcggtgggatgtctcgtttgttccacgggctttaccgcaaccatctcatcaagagcaaattcgccatgaaggatcgcccggtcctattgaacagctgggagggcctaggttttgactacaatgagagcaccatctacaaccttgctcaagaatctgcagacttgggagtcaaactcttcgtcctggatgatggatggttcggtgataagtatcctcgactgtctgacaacgccggtttaggtgactgggtacccaatcccgacaggttcccagacggtctggatcacgcagtgactagtattacggcgctgaaagctgcgaacacatccaccaagctccgatttggtctctggtttgagcctgagatggtcaaccctaattccagcctctatcacgaacaccctgactgggccttacatgccggatcctatccacgcacagaacgacgtaatcagctcgttttaaacgtggctcttccagaggtacaagactttatcatcaagtctgtgtctagtattctgagcagcgccgatatcacctatgtgaagtgggataacaatcgtggtattcatgaaatgccctcgccatccactgaccacgaatacatgctaggcatgtaccgggtattcaacaacttgaccactcaattccctaatgttctgtgggagggctgcgcttcaggtggcggtcgcttcgatgctggtgtactccagtacttcccccagatctggacctctgatgataccgatgccgttgagcgcatcaccattcaaatgggaacctcactcgtgtatcccccgagcgcgatgggtgctcacctttctgccgtccccaaccaacagaccggtaggacactgcctgtcgcattccgtggccacgttgccatgatgggaggctctttcggccttgagctagatcccgccgaaatcccgagtgatgacaaggctgctctgcctggcctcatttcacttgctgagaaggtcaacccaatcatcttgaccggggatatgtaccgcttgaatctaccggaggactcgaattggcccgccgttcaatttatctcgcaagatgcgtcgcaggcggtgctattctacttccagattaaccccaacatcaatcatgcactaccgtggatcaagctgcaaggattggatcccaaggcagtctatagcgtggatggtaatgccacgtattcaggatcagccctgatgaatgttgggttacagtttgtctttgaaacagactacggcagtcaagttgtgttcattgagaagcagtga

SEQ ID NO: 2 - protein, 742 aa, Penicillium pseudopulvillorum
MQKAVASASLLALLGSTSAVAAQSFSNVVVDGTTFALNGDNFSYRFHVDNETGDLWSDHFGASVTGDIPFENVPAVNGWVGMPGRVRREFPDQGRGDFRIPAIRIRQSEGYTVSDLQYQSYDVIQGKPELPGLPATFGTDKDVTTLVVHLYDNYSAVAADLSYSVFPKYDAIVRSVNVTNKGQDNITIEALASLSVDFPYQDLDMISLRGDWAREAHRERRKVEYGIQGFGSSTGYSSHLHNPFLALVDPSATESSGEAWGFSLVYTGSFSVDVEKGSQGFTRALLGLNPNQLSWNLGTGETITTPECVSVYSQNGVGGMSRLFHGLYRNHLIKSKFAMKDRPVLLNSWEGLGFDYNESTIYNLAQESADLGVKLFVLDDGWFGDKYPRLSDNAGLGDWVPNPDRFPDGLDHAVTSITALKAANTSTKLRFGLWFEPEMVNPNSSLYHEHPDWALHAGSYPRTERRNQLVLNVALPEVQDFIIKSVSSILSSADITYVKWDNNRGIHEMPSPSTDHEYMLGMYRVFNNLTTQFPNVLWEGCASGGGRFDAGVLQYFPQIWTSDDTDAVERITIQMGTSLVYPPSAMGAHLSAVPNQQTGRTLPVAFRGHVAMMGGSFGLELDPAEIPSDDKAALPGLISLAEKVNPIILTGDMYRLNLPEDSNWPAVQFISQDASQAVLFYFQINPNINHALPWIKLQGLDPKAVYSVDGNATYSGSALMNVGLQFVFETDYGSQVVFIEKQ

SEQ ID NO: 3 - protein, 721 aa, Penicillium pseudopulvillorum
  mat_peptide (1)..(721)
AQSFSNVVVDGTTFALNGDNFSYRFHVDNETGDLWSDHFGASVTGDIPFENVPAVNGWVGMPGRVRREFPDQGRGDFRIPAIRIRQSEGYTVSDLQYQSYDVIQGKPELPGLPATFGTDKDVTTLVVHLYDNYSAVAADLSYSVFPKYDAIVRSVNVTNKGQDNITIEALASLSVDFPYQDLDMISLRGDWAREAHRERRKVEYGIQGFGSSTGYSSHLHNPFLALVDPSATESSGEAWGFSLVYTGSFSVDVEKGSQGFTRALLGLNPNQLSWNLGTGETITTPECVSVYSQNGVGGMSRLFHGLYRNHLIKSKFAMKDRPVLLNSWEGLGFDYNESTIYNLAQESADLGVKLFVLDDGWFGDKYPRLSDNAGLGDWVPNPDRFPDGLDHAVTSITALKAANTSTKLRFGLWFEPEMVNPNSSLYHEHPDWALHAGSYPRTERRNQLVLNVALPEVQDFIIKSVSSILSSADITYVKWDNNRGIHEMPSPSTDHEYMLGMYRVFNNLTTQFPNVLWEGCASGGGRFDAGVLQYFPQIWTSDDTDAVERITIQMGTSLVYPPSAMGAHLSAVPNQQTGRTLPVAFRGHVAMMGGSFGLELDPAEIPSDDKAALPGLISLAEKVNPIILTGDMYRLNLPEDSNWPAVQFISQDASQAVLFYFQINPNINHALPWIKLQGLDPKAVYSVDGNATYSGSALMNVGLQFVFETDYGSQVVFIEKQ

SEQ ID NO: 4 - protein, 747 aa, Aspergillus niger
MIGSSHAVVALGLFTLYGHSAAAPATGASNSQTIVTNGTSFALNGDNVSYRFHVNSTTGDLISDHFGGVVSGTIPSPVEPAVNGWVGMPGRIRREFPDQGRGDFRIPAVRIRESAGYTVSDLQYVSHEVIEGKNALPGLPATFGDAQAVTTLVVHLYDNYSSVAADLSYSIFPKYDAIVRSVNVINQGPGNITIEALASISIDFPYEDLDMVSLRGDWAREANVQRSKVQYGVQGFGSSTGYSSHLHNPFLAIVDPATTESQGEAWGFNLVYTGSFSAQVEKGSQGFTRALLGFNPDQLSWNLGPGETLTSPECVAVYSDKGLGSVSRKFHRLYRNHLMKSKFATSDRPVLLNSWEGVYFDYNQSSIETLAEESAALGVHLFVMDDGWFGDKYPRVSDNAGLGDWMPNPARFPDGLTPVVQDITNLTVNGTESTKLRFGIWVEPEMVNPNSTLYHEHPEWALHAGPYPRTERRNQLVLNLALPAVQDFIIDFMTNLLQDTGISYVKWDNNRGIHETPSPSTDHQYMLGLYRVFDTLTTRFPDVLWEGCASGGGRFDAGMLQYVPQIWTSDNTDAIDRITIQFGTSLAYPPSAMGAHLSAVPNAQTGRTVPITFRAHVAMMGGSFGLELDPATVEGDEIVPELLALAEKVNPIILNGDLYRLRLPQDSQWPAALFVTQDGAQAVLFYFQVQPNVNHAVPWVRLQGLDPKADYTVDGDQTYSGATLMNLGLQYSFDTEYGSKVVFLERQ